European Patent Application EP 4 268 890 A1, published November 1, 2023. Title: Methylglyoxal-scavenging cyclic peptides and their use for the prevention and treatment of diseases associated with elevated methylglyoxal levels. Applicant: Universität Heidelberg. The sequence listing filed with the application follows.

SEQUENCE LISTING (4 sequences)

SEQ ID NO: 1 - protein, 6 aa, Artificial Sequence
  Amino acid sequence of cyclic peptide
KKKKKE

SEQ ID NO: 2 - protein, 6 aa, Artificial Sequence
  Amino acid sequence of cyclic peptide
KKEKKE

SEQ ID NO: 3 - protein, 6 aa, Artificial Sequence
  Amino acid sequence of cyclic peptide
KKEKEE

SEQ ID NO: 4 - protein, 7 aa, Artificial Sequence
  Amino acid sequence of cyclic peptide
KEKEKKE